European Patent Application EP 4 212 173 A1, published July 19, 2023. Title: Vaccine composition for chicken pox or herpes zoster and method using the same. Applicant: EUBIOLOGICS CO.,LTD. The sequence listing filed with the application follows.

SEQUENCE LISTING (24 sequences)

SEQ ID NO: 1 - protein, 526 aa, Artificial Sequence
  gEs
MKWVTFISLLFLFSSAYSSVLRYDDFHTDEDKLDTNSVYEPYYHSDHAESSWVNRGESSRKAYDHNSPYIWPRNDYDGFLENAHEHHGVYNQGRGIDSGERLMQPTQMSAQEDLGDDTGIHVIPTLNGDDRHKIVNVDQRQYGDVFKGDLNPKPQGQRLIEVSVEENHPFTLRAPIQRIYGVRYTETWSFLPSLTCTGDAAPAIQHICLKHTTCFQDVVVDVDCAENTKEDQLAEISYRFQGKKEADQPWIVVNTSTLFDELELDPPEIEPGVLKVLRTEKQYLGVYIWNMRGSDGTSTYATFLVTWKGDEKTRNPTPAVTPQPRGAEFHMWNYHSHVFSVGDTFSLAMHLQYKIHEAPFDLLLEWLYVPIDPTCQPMRLYSTCLYHPNAPQCLSHMNSGCTFTSPHLAQRVASTVYQNCEHADNYTAYCLGISHMEPSFGLILHDGGTTLKFVDTPESLSGLYVFVVYFNGHVEAVAYTVVSTVDHFVNAIEERGFPPTAGQPPATTKPKEITPVNPGTSPLIRY

SEQ ID NO: 2 - protein, 534 aa, Artificial Sequence
  gEt
MKWVTFISLLFLFSSAYSSVLRYDDFHTDEDKLDTNSVYEPYYHSDHAESSWVNRGESSRKAYDHNSPYIWPRNDYDGFLENAHEHHGVYNQGRGIDSGERLMQPTQMSAQEDLGDDTGIHVIPTLNGDDRHKIVNVDQRQYGDVFKGDLNPKPQGQRLIEVSVEENHPFTLRAPIQRIYGVRYTETWSFLPSLTCTGDAAPAIQHICLKHTTCFQDVVVDVDCAENTKEDQLAEISYRFQGKKEADQPWIVVNTSTLFDELELDPPEIEPGVLKVLRTEKQYLGVYIWNMRGSDGTSTYATFLVTWKGDEKTRNPTPAVTPQPRGAEFHMWNYHSHVFSVGDTFSLAMHLQYKIHEAPFDLLLEWLYVPIDPTCQPMRLYSTCLYHPNAPQCLSHMNSGCTFTSPHLAQRVASTVYQNCEHADNYTAYCLGISHMEPSFGLILHDGGTTLKFVDTPESLSGLYVFVVYFNGHVEAVAYTVVSTVDHFVNAIEERGFPPTAGQPPATTKPKEITPVNPGTSPLIRYAAWTGGLA

SEQ ID NO: 3 - DNA, 1581 bp, Artificial Sequence
  gEs
atgaagtgggtgacatttatctctctgcttttcctgttcagcagcgcctacagtagcgtgctgcgctacgacgatttccacatcgacgaggataagctggacaccaatagcgtgtatgagccttactatcactctgatcatgccgagtccagctgggtgaacaggggcgagtcttcccggaaggcttacgaccacaactctccctatatctggcccaggaatgactacgatggctttctggagaacgcccatgagcaccatggcgtgtataatcagggccggggcatcgactctggcgagagactgatgcagcctacacagatgtccgctcaggaggatctgggcgacgatacaggcatccacgtgatcccaaccctgaatggcgacgatcgccataagatcgtgaacgtggatcagaggcagtacggcgacgtgttcaagggcgatctgaatccaaagccccagggccagcggctgatcgaggtgtccgtggaggagaaccatccattcaccctgagagcccccatccagcgcatctacggcgtgaggtataccgagacatggtcctttctgcctagcctgacctgcacaggcgacgctgctccagctatccagcacatctgcctgaagcataccacatgttttcaggacgtggtggtggacgtggattgtgccgagaatacaaaggaggatcagctggctgagatcagctacagattccagggcaagaaggaggccgatcagccatggatcgtggtgaacacctctacactgtttgacgagctggagctggacccccccgagatcgagccaggcgtgctgaaggtgctgcgcaccgagaagcagtacctgggcgtgtatatctggaacatgaggggctctgacggcacctccacatacgctaccttcctggtgacatggaagggcgatgagaagacccggaatccaacaccagctgtgacccctcagccaagaggcgctgagtttcacatgtggaactatcacagccacgtgttctccgtgggcgacaccttttccctggccatgcacctgcagtacaagatccatgaggctccattcgacctgctgctggagtggctgtatgtgcccatcgatcctacatgccagcccatgcggctgtacagcacctgtctgtatcacccaaatgccccccagtgcctgtcccatatgaacagcggctgtacctttacatccccacacctggcccagagagtggcctccacagtgtaccagaactgcgagcatgccgacaattacaccgcttattgtctgggcatctctcacatggagccctccttcggcctgatcctgcatgacggcggcaccacactgaagtttgtggatacacctgagagcctgtctggcctgtacgtgttcgtggtgtacttcaacggccacgtggaggccgtggcttatacagtggtgtctaccgtggatcatttcgtgaacgctatcgaggagaggggatttccaccaaccgctggacagcctccagctaccacaaagcccaaggagatcacacctgtgaacccaggcacctcccctctgattcgttattga

SEQ ID NO: 4 - DNA, 1605 bp, Artificial Sequence
  gEt
atgaagtgggtgacatttatctctctgcttttcctgttcagcagcgcctacagtagcgtgctgcgctacgacgatttccacatcgacgaggataagctggacaccaatagcgtgtatgagccttactatcactctgatcatgccgagtccagctgggtgaacaggggcgagtcttcccggaaggcttacgaccacaactctccctatatctggcccaggaatgactacgatggctttctggagaacgcccatgagcaccatggcgtgtataatcagggccggggcatcgactctggcgagagactgatgcagcctacacagatgtccgctcaggaggatctgggcgacgatacaggcatccacgtgatcccaaccctgaatggcgacgatcgccataagatcgtgaacgtggatcagaggcagtacggcgacgtgttcaagggcgatctgaatccaaagccccagggccagcggctgatcgaggtgtccgtggaggagaaccatccattcaccctgagagcccccatccagcgcatctacggcgtgaggtataccgagacatggtcctttctgcctagcctgacctgcacaggcgacgctgctccagctatccagcacatctgcctgaagcataccacatgttttcaggacgtggtggtggacgtggattgtgccgagaatacaaaggaggatcagctggctgagatcagctacagattccagggcaagaaggaggccgatcagccatggatcgtggtgaacacctctacactgtttgacgagctggagctggacccccccgagatcgagccaggcgtgctgaaggtgctgcgcaccgagaagcagtacctgggcgtgtatatctggaacatgaggggctctgacggcacctccacatacgctaccttcctggtgacatggaagggcgatgagaagacccggaatccaacaccagctgtgacccctcagccaagaggcgctgagtttcacatgtggaactatcacagccacgtgttctccgtgggcgacaccttttccctggccatgcacctgcagtacaagatccatgaggctccattcgacctgctgctggagtggctgtatgtgcccatcgatcctacatgccagcccatgcggctgtacagcacctgtctgtatcacccaaatgccccccagtgcctgtcccatatgaacagcggctgtacctttacatccccacacctggcccagagagtggcctccacagtgtaccagaactgcgagcatgccgacaattacaccgcttattgtctgggcatctctcacatggagccctccttcggcctgatcctgcatgacggcggcaccacactgaagtttgtggatacacctgagagcctgtctggcctgtacgtgttcgtggtgtacttcaacggccacgtggaggccgtggcttatacagtggtgtctaccgtggatcatttcgtgaacgctatcgaggagaggggatttccaccaaccgctggacagcctccagctaccacaaagcccaaggagatcacacctgtgaacccaggcacctcccctctgattcgttatgctgcttggacagggggtctggcatga

SEQ ID NO: 5 - protein, 623 aa, Human herpesvirus 3
MGTVNKPVVGVLMGFGIITGTLRITNPVRASVLRYDDFHTDEDKLDTNSVYEPYYHSDHAESSWVNRGESSRKAYDHNSPYIWPRNDYDGFLENAHEHHGVYNQGRGIDSGERLMQPTQMSAQEDLGDDTGIHVIPTLNGDDRHKIVNVDQRQYGDVFKGDLNPKPQGQRLIEVSVEENHPFTLRAPIQRIYGVRYTETWSFLPSLTCTGDAAPAIQHICLKHTTCFQDVVVDVDCAENTKEDQLAEISYRFQGKKEADQPWIVVNTSTLFDELELDPPEIEPGVLKVLRTEKQYLGVYIWNMRGSDGTSTYATFLVTWKGDEKTRNPTPAVTPQPRGAEFHMWNYHSHVFSVGDTFSLAMHLQYKIHEAPFDLLLEWLYVPIDPTCQPMRLYSTCLYHPNAPQCLSHMNSGCTFTSPHLAQRVASTVYQNCEHADNYTAYCLGISHMEPSFGLILHDGGTTLKFVDTPESLSGLYVFVVYFNGHVEAVAYTVVSTVDHFVNAIEERGFPPTAGQPPATTKPKEITPVNPGTSPLIRYAAWTGGLAAVVLLCLVIFLICTAKRMRVKAYRVDKSPYNQSMYYAGLPVDDFEDSESTDTEEEFGNAIGGSHGGSSYTVYIDKTR

SEQ ID NO: 6 - protein, 18 aa, Artificial Sequence
  mutant signal peptide
MKWVTFISLLFLFSSAYS

SEQ ID NO: 7 - DNA, 1659 bp, Artificial Sequence
  codon optimized nucleic acid sequence encoding 1-546 amino acids of gE antigen with 6 histidine
atgggaactgtgaacaagcccgtcgtgggggtcctgatgggtttcggtattattactggaactctgcgtattacaaatcctgtccgtgccagcgtgctgcgctacgacgatttccacatcgacgaggataagctggacaccaatagcgtgtatgagccttactatcactctgatcatgccgagtccagctgggtgaacaggggcgagtcttcccggaaggcttacgaccacaactctccctatatctggcccaggaatgactacgatggctttctggagaacgcccatgagcaccatggcgtgtataatcagggccggggcatcgactctggcgagagactgatgcagcctacacagatgtccgctcaggaggatctgggcgacgatacaggcatccacgtgatcccaaccctgaatggcgacgatcgccataagatcgtgaacgtggatcagaggcagtacggcgacgtgttcaagggcgatctgaatccaaagccccagggccagcggctgatcgaggtgtccgtggaggagaaccatccattcaccctgagagcccccatccagcgcatctacggcgtgaggtataccgagacatggtcctttctgcctagcctgacctgcacaggcgacgctgctccagctatccagcacatctgcctgaagcataccacatgttttcaggacgtggtggtggacgtggattgtgccgagaatacaaaggaggatcagctggctgagatcagctacagattccagggcaagaaggaggccgatcagccatggatcgtggtgaacacctctacactgtttgacgagctggagctggacccccccgagatcgagccaggcgtgctgaaggtgctgcgcaccgagaagcagtacctgggcgtgtatatctggaacatgaggggctctgacggcacctccacatacgctaccttcctggtgacatggaagggcgatgagaagacccggaatccaacaccagctgtgacccctcagccaagaggcgctgagtttcacatgtggaactatcacagccacgtgttctccgtgggcgacaccttttccctggccatgcacctgcagtacaagatccatgaggctccattcgacctgctgctggagtggctgtatgtgcccatcgatcctacatgccagcccatgcggctgtacagcacctgtctgtatcacccaaatgccccccagtgcctgtcccatatgaacagcggctgtacctttacatccccacacctggcccagagagtggcctccacagtgtaccagaactgcgagcatgccgacaattacaccgcttattgtctgggcatctctcacatggagccctccttcggcctgatcctgcatgacggcggcaccacactgaagtttgtggatacacctgagagcctgtctggcctgtacgtgttcgtggtgtacttcaacggccacgtggaggccgtggcttatacagtggtgtctaccgtggatcatttcgtgaacgctatcgaggagaggggatttccaccaaccgctggacagcctccagctaccacaaagcccaaggagatcacacctgtgaacccaggcacctcccctctgattcgttatgctgcttggacagggggtctggcacaccaccaccaccaccactga

SEQ ID NO: 8 - DNA, 31 bp, Artificial Sequence
  forward primer 1
gctagcgccgccaccatgggaactgtgaaca

SEQ ID NO: 9 - DNA, 30 bp, Artificial Sequence
  reverse primer 1
gcggccgcttatcagtggtggtggtggtgg

SEQ ID NO: 10 - DNA, 33 bp, Artificial Sequence
  reverse primer 2
gaattctcattatgccagaccccctgtccaagc

SEQ ID NO: 11 - DNA, 30 bp, Artificial Sequence
  reverse primer 3
gtaccggatcagaggggaggtgcctgggtt

SEQ ID NO: 12 - DNA, 30 bp, Artificial Sequence
  forward primer 1
gctagcgccgccaccatgggaactgtgaac

SEQ ID NO: 13 - DNA, 49 bp, Artificial Sequence
  reverse primer 4
gcggccgctcaatggtgatggtgatgatgataacgaatcagaggggagg

SEQ ID NO: 14 - DNA, 21 bp, Artificial Sequence
  forward primer 3
agcgtgctgcgctacgacgat

SEQ ID NO: 15 - DNA, 90 bp, Artificial Sequence
  forward primer 4
aagcttgccgccaccatgaagtgggtgacatttatctctctgcttttcctgttcagcagcgcctacagtagcgtgctgcgctacgacgat

SEQ ID NO: 16 - DNA, 30 bp, Artificial Sequence
  forward primer 5
aagcttgccgccaccatgaagtgggtgaca

SEQ ID NO: 17 - DNA, 33 bp, Artificial Sequence; identical to SEQ ID NO: 10
  reverse primer 5

SEQ ID NO: 18 - DNA, 33 bp, Artificial Sequence
  reverse primer 6
gaattctcattaataacgaatcagaggggaggt

SEQ ID NO: 19 - DNA, 21 bp, Artificial Sequence
  CMV-F1 (vector) primer
cgcaaatgggcggtaggcgtg

SEQ ID NO: 20 - DNA, 21 bp, Artificial Sequence
  VZV-F2-403 primer
caggcatccacgtgatcccaa

SEQ ID NO: 21 - DNA, 21 bp, Artificial Sequence
  VZV-F3-1053 primer
tatcacagccacgtgttctcc

SEQ ID NO: 22 - DNA, 18 bp, Artificial Sequence
  VZV-R1~600 primer
ccatgtctcggtatacct

SEQ ID NO: 23 - DNA, 17 bp, Artificial Sequence
  VZV-R2~1200 primer
tgggtgatacagacagg

SEQ ID NO: 24 - DNA, 18 bp, Artificial Sequence
  VZV-R3 plus 150 (vector) primer
agagtgccagccctggga